European Patent Application EP 4 144 833 A1, published March 8, 2023. Title: Strain of Lactobacillus crispatus Capable of Preventing and/or Treating Helicobacter pylori Infection. Applicant: Jiangnan University. The sequence listing filed with the application follows.

SEQUENCE LISTING (1 sequence)

SEQ ID NO: 1 - DNA, 1165 bp, Artificial Sequence
  Synthetic DNA
  misc_feature (4)..(9): n is a, c, g, or t
  misc_feature (11)..(11): n is a, c, g, or t
  misc_feature (13)..(14): n is a, c, g, or t
  misc_feature (1082)..(1082): n is a, c, g, or t
  misc_feature (1087)..(1087): n is a, c, g, or t
  misc_feature (1151)..(1151): n is a, c, g, or t
  misc_feature (1154)..(1158): n is a, c, g, or t
  misc_feature (1164)..(1165): n is a, c, g, or t
gagnnnnnntncnngccttagacggctccttcccgaaggttaggccaccggctttgggcattgcagactcccatggtgtgacgggcggtgtgtacaaggcccgggaacgtattcaccgcggcgtgctgatccgcgattactagcgattccagcttcgtgcagtcgagttgcagactgcagtccgaactgagaacagctttcagagattcgcttgccttcgcaggctcgcttctcgttgtactgcccattgtagcacgtgtgtagcccaggtcataaggggcatgatgacttgacgtcatccccaccttcctccggtttgtcaccggcagtctcattagagtgcccaacttaatgctggcaactaataacaagggttgcgctcgttgcgggacttaacccaacatctcacgacacgagctgacgacagccatgcaccacctgtcttagcgtccccgaagggaactttgtatctctacaaatggcactagatgtcaagacctggtaaggttcttcgcgttgcttcgaattaaaccacatgctccaccgcttgtgcgggcccccgtcaattcctttgagtttcaaccttgcggtcgtactccccaggcggagtgcttaatgcgttagctacagcactgagaggcggaaacctcccaacacttagcactcatcgtttacggcatggactaccagggtatctaatcctgttcgctacccatgctttcgagcctcagcgtcagttgcagaccagagagccgccttcgccactggtgttcttccatatatctacgcattccaccgctacacatggagttccactctcctcttctgcactcaagaaaaacagtttccgatgcagttcctcggttaagccgagggctttcacatcagacttattcttccgcctgcgctcgctttacgcccaataaatccggacaacgcttgccacctacgtattaccgcggctgctggcacgtagttagccgtgactttctggttgattaccgtcaaataaaggccagttactacctctatccttcttcaccaacaacagagctttacgatccgaaaacctctcactcacncggcntgctccatcagacttgcgtcattgtggaagattccctactgctgcctccgtagaagttggggcngtnnnnnctcagnn